European Patent Application EP 4 582 553 A1, published July 9, 2025. Title: 一管式RT-qPCR全预混反应试剂、应用及RT-qPCR方法. Applicant: 上海伯杰医疗科技股份有限公司. Application CN. The sequence listing filed with the application follows.

SEQUENCE LISTING (20 sequences)

SEQ ID NO: 1 - protein, 118 aa, synthetic construct
DIEMTQSSGAELARPGASVKMSCKASGTFRYSDYMHWVKQRPGQGLEWIGYRGPNDRYTKYNQKFKKATLTADKSSSTAYMQLSSLTSEDSAVYYCGRDDYYCSHDATWGQGTTLSRT

SEQ ID NO: 2 - protein, 105 aa, synthetic construct
VQLVESGGMSASPGEKVTMTCAASSVYSSMHWYQQKSGTSPKRWIYDYQKLASGVPARFSGSGSGTSYSLTISSMEAETPETYYCEDWNPSDTFFGSGTTISRDN

SEQ ID NO: 3 - DNA, 19 bp, synthetic construct
  source 1..19: mol_type = other DNA
ctggtggattggaaatgta

SEQ ID NO: 4 - DNA, 18 bp, synthetic construct
  source 1..18: mol_type = other DNA
aattcgggcagaagattg

SEQ ID NO: 5 - DNA, 21 bp, synthetic construct
  source 1..21: mol_type = other DNA
ctgtccacaatccgaggtcat

SEQ ID NO: 6 - DNA, 18 bp, synthetic construct
  source 1..18: mol_type = other DNA
agtcttctaaccgaggtc

SEQ ID NO: 7 - DNA, 18 bp, synthetic construct
  source 1..18: mol_type = other DNA
tcgagatctgcgttcttc

SEQ ID NO: 8 - DNA, 21 bp, synthetic construct
  source 1..21: mol_type = other DNA
catcctcaagtctctgtgcga

SEQ ID NO: 9 - DNA, 19 bp, synthetic construct
  source 1..19: mol_type = other DNA
ggagtcttatcccaatttg

SEQ ID NO: 10 - DNA, 18 bp, synthetic construct
  source 1..18: mol_type = other DNA
cttctgtgaccagtctaa

SEQ ID NO: 11 - DNA, 24 bp, synthetic construct
  source 1..24: mol_type = other DNA
caagagcaccgattatcaccagaa

SEQ ID NO: 12 - DNA, 19 bp, synthetic construct
  source 1..19: mol_type = other DNA
gcaagtagtcacagattag

SEQ ID NO: 13 - DNA, 19 bp, synthetic construct
  source 1..19: mol_type = other DNA
gattcttgtcactagcatt

SEQ ID NO: 14 - DNA, 19 bp, synthetic construct
  source 1..19: mol_type = other DNA
taccagcactacaagccgc

SEQ ID NO: 15 - DNA, 18 bp, synthetic construct
  source 1..18: mol_type = other DNA
cacaggtgagcagtcatc

SEQ ID NO: 16 - DNA, 18 bp, synthetic construct
  source 1..18: mol_type = other DNA
cgccctactgaagaaact

SEQ ID NO: 17 - DNA, 20 bp, synthetic construct
  source 1..20: mol_type = other DNA
tacaggcaaggttccagcac

SEQ ID NO: 18 - DNA, 18 bp, synthetic construct
  source 1..18: mol_type = other DNA
cttccagagattcgtttg

SEQ ID NO: 19 - DNA, 19 bp, synthetic construct
  source 1..19: mol_type = other DNA
catattattcgggcattga

SEQ ID NO: 20 - DNA, 19 bp, synthetic construct
  source 1..19: mol_type = other DNA
cagacagccaccaacccat